European Patent Specification EP 3 762 479 B1, published August 19, 2026. Title: HIGHLY MULTIPLEXED PHYLOGENETIC IMAGING OF MICROBIAL COMMUNITIES. Applicant: Cornell University. The sequence listing filed with the application follows.

SEQUENCE LISTING (17 sequences)

SEQ ID NO: 1 - DNA, 20 bp, Artificial Sequence
  Oligonucleotide
tatccttcaatccctccaca

SEQ ID NO: 2 - DNA, 20 bp, Artificial Sequence
  Oligonucleotide
acactaccaccatttcctat

SEQ ID NO: 3 - DNA, 20 bp, Artificial Sequence
  Oligonucleotide
actccactactactcactct

SEQ ID NO: 4 - DNA, 20 bp, Artificial Sequence
  Oligonucleotide
accctctaacttccatcaca

SEQ ID NO: 5 - DNA, 20 bp, Artificial Sequence
  Oligonucleotide
accacaacccattcctttca

SEQ ID NO: 6 - DNA, 20 bp, Artificial Sequence
  Oligonucleotide
tttactccctacacctccaa

SEQ ID NO: 7 - DNA, 20 bp, Artificial Sequence
  Oligonucleotide
accctttacaaacacaccct

SEQ ID NO: 8 - DNA, 20 bp, Artificial Sequence
  Oligonucleotide
tcctattctcaacctaacct

SEQ ID NO: 9 - DNA, 20 bp, Artificial Sequence
  Oligonucleotide
ttctccctctatcaactcta

SEQ ID NO: 10 - DNA, 20 bp, Artificial Sequence
  Oligonucleotide
acccttactactacatcatc

SEQ ID NO: 11 - DNA, 107 bp, Artificial Sequence
  Oligonucleotide
cgatgcgccaattccggttctgtggagggattgaaggataaatctctcgcgagttcgcaactcgaaccaacccgcgagcgatgatcagtctattttcttatccgacg

SEQ ID NO: 12 - DNA, 106 bp, Artificial Sequence
  Oligonucleotide
cgatgcgccaattccggttcataggaaatggtggtagtgtatggccgcgggatcatccagaagactcaacccgcgagcgatgatcagtctattttcttatccgacg

SEQ ID NO: 13 - DNA, 106 bp, Artificial Sequence
  Oligonucleotide
cgatgcgccaattccggttcataggaaatggtggtagtgtgagattcaaccgcgcgaagcccgttctgtggagggattgaaggatacaacccgcgagcgatgatca

SEQ ID NO: 14 - DNA, 20 bp, Artificial Sequence
  Oligonucleotide
agagtttgatcmtggctcag

SEQ ID NO: 15 - DNA, 22 bp, Artificial Sequence
  Oligonucleotide
tacggytaccttgttacgactt

SEQ ID NO: 16 - DNA, 20 bp, Artificial Sequence
  Oligonucleotide
cgatgcgccaattccggttc

SEQ ID NO: 17 - DNA, 20 bp, Artificial Sequence
  Oligonucleotide
gtctattttcttatccgacg